European Patent Specification EP 3 068 794 B1, published September 13, 2023. Title: Methods of Modulating Seed and Organ Size in Plants. Applicant: Plant Bioscience Limited. The sequence listing filed with the application follows.

SEQUENCE LISTING (54 sequences)

SEQ ID NO: 1 - protein, 66 aa, Artificial sequence
  Synthetic sequence: LIM domain
  VARIANT (2)..(3): Xaa is any amino acid
  VARIANT (5)..(27): Xaa at positions 5 to 27 is any amino acid and up to seven of them may be absent; represents a range of 16 - 23 amino acids.
  VARIANT (28)..(28): Xaa is His or Cys
  VARIANT (29)..(32): Xaa at positions 29 to 32 is any amino acid and any two of them may be absent; represents a string of 2 or 4 amino acids.
  VARIANT (33)..(33): Xaa is Cys, His or Glu
  VARIANT (34)..(35): Xaa is any amino acid
  VARIANT (37)..(38): Xaa is any amino acid
  VARIANT (40)..(60): Xaa at positions 40 to 60 is any amino acid and up to seven of them may be absent; represents a range of 14 - 21 amino acids.
  VARIANT (61)..(61): Xaa is Cys or His
  VARIANT (62)..(64): Xaa at positions 62 - 64 is any amino acid and any one or two of them may be absent; represents a string of 2 or 1 or 3 amino acids.
  VARIANT (65)..(65): Xaa is Cys, His, Asp or Glu
  VARIANT (66)..(66): Xaa is any amino acid
CXXCXXXXXXXXXXXXXXXXXXXXXXXXXXXXXXXCXXCXXXXXXXXXXXXXXXXXXXXXXXXXXX

SEQ ID NO: 2 - protein, 63 aa, Artificial sequence
  Synthetic sequence: LIM domain
  VARIANT (2)..(3): Xaa is any amino acid
  VARIANT (5)..(27): Xaa at positions 5 - 27 is any amino acid and up to seven of them may be absent; represents a range of 16 - 23 amino acids.
  VARIANT (29)..(30): Xaa is any amino acid
  VARIANT (32)..(33): Xaa is any amino acid
  VARIANT (35)..(36): Xaa is any amino acid
  VARIANT (38)..(58): Xaa at positions 38 to 58 is any amino acid and up to seven of them may be absent; represents a range of 14 - 21 amino acids.
  VARIANT (60)..(61): Xaa is any amino acid
  VARIANT (63)..(63): Xaa is any amino acid
CXXCXXXXXXXXXXXXXXXXXXXXXXXHXXCXXCXXCXXXXXXXXXXXXXXXXXXXXXHXXCX

SEQ ID NO: 3 - protein, 53 aa, Arabidopsis thaliana
CAGCNMEIGHGRFLNCLNSLWHPECFRCYGCSQPISEYEFSTSGNYPFHKACY

SEQ ID NO: 4 - protein, 504 aa, Setaria italica
MGWLSKIFKGSVNRVSRGHYNGNSHEGYSTQHTKSYGAHGNEDEDMDHAIALSLSEQDQRKGKAIDTEHHLDEDEQLARALQENTSPTLDEDEQLARALQESMNDEHPPRQHIPIEDVHSESAPASSLPPYVFPTNGSRVCAGCKTPIGQGRFLSCMDSVWHPQCFRCYGCDIPISEYEFAVHEDHAYHRSCYKERFHPKCDVCNSFIPTNKNGLIEYRAHPFWMQKYCPSHENDGTPRCCSCERMEPKHSQYITLDDGRRLCLECLHTAIMDTNECQPLYIDIQEFYEGMNMKVEQQVPLLLVERQALNEAMEAEKIGHHLPETRGLCLSEEQIVRTILRRPIIGPGNRIIDMITGPYKLVRRCEVTAILILYGLPRLLTGSILAHEMMHAYLRLKGYRTLSPEVEEGICQVLAHLWLESEITSGSGSMATTSAASSSSSTSSSSKKGAKTEFEKRLGEFFKHQIETDPSVAYGDGFRAGMRAVERYGLRSTLDHIKLTGSFP

SEQ ID NO: 5 - protein, 487 aa, Brachypodium distachyon
MGWLNKIFKGSVNRVSRGNYDGNWHDGNSSENIRGAYDESDNEDIDRAIALSLAEEDPNKGKAIIDPDYSLEEDEQLARALHESLNTGSPPHQNVPVVDVPSERVPTREPPPPVFLSSGFRACAGCNNPIGNGRFLSCMDSVWHPQCFRCFACNKPISEYEFAMHENQPYHKSCYKDFFHPKCDVCKDFIPTNKDGLIEYRAHPFWMQKYCPSHEDDGTPRCCSCERMEPTDIKYIRLDDGRKLCLECLTSATMDSPECQHLYMDIQEFFEGLNMKVEQQVPLLLVERQALNEALEAEKSGHHLPETRGLCLSEEQIVRTILRRPTIGPGNRIIDMITGPYKLVRRCEVTAILILYGLPRLQTGSILAHEMMHAYLRLKGYRSLSPQVEEGICQVLSHMWLESEIIAGASGNTASTSVPSSSSAPTSSKKGAKTEFEKRLGAFIKNQIETDSSVEYGDGFRAGNRAVERYGLRSTLDHMKITGSFPY

SEQ ID NO: 6 - protein, 514 aa, Brassica rapa
MGWLNKIFKGSNQRHPLGNEHYHHNGGYYENYPHEHSEPSAETDADHTQEPSTSEEETWNGKENEEVDRVIALSILEEENQRPETNTGAWKHAMMDDDEQLARAIQESMIARNGTTYDFGNAYGNGHMHGGGNVYDNGDIYYPRPIAFSMDFRICAGCNMEIGHGRYLNCLNALWHPQCFRCYGCSHPISEYEFSTSGNYPFHKACYRERFHPKCDVCSLFISTNHAGLIEYRAHPFWVQKYCPSHEHDATPRCCSCERMEPRNTGYFELNDGRKLCLECLDSSVMDTFQCQPLYLQIQEFYEGLNMTVEQEVPLLLVERQALNEAREGERNGHYHMPETRGLCLSEEQTVRTVRKRSKGNWSGNMITEQFKLTRRCEVTAILILFGLPRLLTGSILAHEMMHAWMRLKGFRPLSQDVEEGICQVMAHKWLEAELAAGSRNSNAASSSSSSYGGVKKGPRSQYERKLGEFFKHQIESDASPVYGDGFRAGRLAVNKYGLWRTLEHIQMTGRFPV

SEQ ID NO: 7 - protein, 532 aa, Brassica rapa
MGWFNKIFKGSTQRFRLGNDHDHNGYYQSYPHDEPSADTDPDPDPDPDETHTQEPSTSEEDTSGQENEDIDRAIALSLIENSQGQTNNTCAANAGKYAMVDEDEQLARAIQESMVVGNTPRQKHGSSYDIGNAYGAGDVYGNGHMHGGGNVYANGDIYYPRPTAFPMDFRICAGCNMEIGHGRYLNCLNALWHPECFRCYGCRHPISEYEFSTSGNYPFHKACYRERYHPKCDVCSLFIPTNHAGLIGYRAHPFWVQKYCPSHEHDATPRCCSCERMEPRNTGYVELNDGRKLCLECLDSAVMDTFQCQPLYLQIQEFYEGLFMKVEQDVPLLLVERQALNEAREGEKNGHYHMPETRGLCLSEEQTVSTVRKRSKHGTGNWAGNMITEPYKLTRQCEVTAILILFGLPRLLTGSILAHEMMHAWMRLKGFRTLSQDVEEGICQVMAHKWLEAELAAGSRNSNVASSSSSRGVKKGPRSQYERKLGEFFKHQIESDASPVYGDGFRAGRLAVNKYGLPKTLEHIQMTGRFPV

SEQ ID NO: 8 - protein, 532 aa, Arabidopsis thaliana
MGWFNKIFKGSNQRLRVGNNKHNHNVYYDNYPTASHDDEPSAADTDADNDEPHHTQEPSTSEDNTSNDQENEDIDRAIALSLLEENQEQTSISGKYSMPVDEDEQLARALQESMVVGNSPRHKSGSTYDNGNAYGAGDLYGNGHMYGGGNVYANGDIYYPRPITFQMDFRICAGCNMEIGHGRFLNCLNSLWHPECFRCYGCSQPISEYEFSTSGNYPFHKACYRERYHPKCDVCSHFIPTNHAGLIEYRAHPFWVQKYCPSHEHDATPRCCSCERMEPRNTRYVELNDGRKLCLECLDSAVMDTMQCQPLYLQIQNFYEGLNMKVEQEVPLLLVERQALNEAREGEKNGHYHMPETRGLCLSEEQTVSTVRKRSKHGTGKWAGNITEPYKLTRQCEVTAILILFGLPRLLTGSILAHEMMHAWMRLKGFRTLSQDVEEGICQVMAHKWLDAELAAGSTNSNAASSSSSSQGLKKGPRSQYERKLGEFFKHQIESDASPVYGDGFRAGRLAVHKYGLRKTLEHIQMTGRFPV

SEQ ID NO: 9 - protein, 478 aa, Theobroma cacao
MDWIKKIFKGCAHKFSEGHHHGNYVEDPHPQFNAPSVSGDAWQELENEDVDRAIALSLLGESQKGRKVIDDEYQLEEDEQLARALQESLNFEPPPQYENANMYQPMPVHFPMGYRICAGCNTEIGHGRFLNCLNAFWHPECFRCHACNLPISDYEFSMSGNYRFHKSCYKERYHPKCDVCNDFIPTNPAGLIEYRAHPFWIQKYCPSHEHDSTPRCCSCERMEPQDTGYVALNDGRKLCLECLDSAVMDTKQCQPLYLDILEFYEGLNMKVEQQVPLLLVERQALNEAREGEKNGHYHMPETRGLCLSEEQTVSTILRQPRFGTGNRAMDMITEPCKLTRRCEVTAILILYGLPRLLTGSILAHEMMHAWMRLQGFRTLSQDVEEGICQVLAHMWLLTQLEYASSSNVASASSSASSRLQKGKRPQFEGKLGEFFKHQIESDTSPVYGDGFRAGHQAVYKYGLRRTLEHIRMTGRFPY

SEQ ID NO: 10 - protein, 474 aa, Glycine max
MGWLSRIFKGSDHNKLSEGHYYKEDAGYYLPSTSGVTNNQNENEDIDRAIALSLVEESRRANNNVNGERILSLQTLLEEDEQLARAIEQSLNLESPPRYGNENMYQPPIQYFPLGICAGCYTEIGFGRYLNCLNAFWHPECFRCRACNLPISDYEFSTSGNYPYHKSCYKESYHPKCDVCKHFIPTNPAGLIEYRAHPFWIQKYCPTHEHDGTPRCCSCERMESQEAGYIALKDGRKLCLECLDSSIMDTNECQPLHADIQRFYDSLNMKLDQQIPLLLVERQALNEAREGEKNGHYHMPETRGLCLSEELSTFSRRPRLGTAMDMRAQPYRPTTRCDVTAILVLYGLPRLLTGSILAHEMMHAWLRLKGYRTLSQDVEEGICQVLAHMWLESELSSASGSNFVSASSSSASHTSRKGKRPQFERKLGEFFKHQIESDISPVYGDGFRAGQKAVRKYGLQRTLHHIRMTGTFPY

SEQ ID NO: 11 - protein, 478 aa, Glycine max
MGWLSRIFKGSDHNKLSEGHYYKEDAGYYLPSTSGVTNDAWNQSQNQNENEDIDRAIALSLVEETQKANNNVNDYRSQLEEDEQLARAIEQSLNLESPPRYGNENMYQPPIQYFPMGSRICAGCYTEIGYGRYLNCLNAFWHPECFRCRACNLPISDYEFSTSGNYPYHKSCYKESYHPKCDVCKHFIPTNPAGLIEYRAHPFWIQKYCPTHEHDGTTRCCSCERMESQEAGYIALKDGRKLCLECLDSAIMDTNECQPLHADIQRFYESLNMKLDQQIPLLLVERQALNEAREGEKNGHYHMPETRGLCLSEELSTFSRRPRLGTTMDMRAQPYRPTTRCDVTAILILYGLPRLLTGSILAHEMMHAWLRLKGYRTLSQDVEEGICQVLSHMWLESELSSASGSNFVSASSSSASHTSRKGKRPQFERKLGEFFKHQIESDISPVYGGGFRAGQKAVSKYGLQRTLHHIRMTGTFPY

SEQ ID NO: 12 - protein, 462 aa, Vitis vinifera
MGWLNKIFKGSSHKISEGNYHGRYQGDTVQNEPSCSGDVWAETENEDIDRAIALSLSEEEQKGKKVIDNEFQLEEDEQLARAIQESLNIESPPQHGNGNGNGNIYQPIPFPYSTGFRICAGCNTEIGHGRFLSCMGAVWHPECFRCHGCGYPISDYEYSMNGNYPYHKSCYKEHYHPKCDVCKHFIPTNPAGLIEYRAHPFWVQKYCPSHEHDRTPRCCSCERMEPRDTRYVALNDGRKLCLECLDSAIMDTNECQPLYLDIQEFYEGLNMKVQQQVPLLLVERQALNEAMEGEKSGHHHMPETRGLCLSEEQTVSTILRRPKIGTGNRVMNMITEPCKLTRRCDVTAVLILYGLPRLLTGSILAHEMMHAWLRLNGYRTLAQDVEEGICQVLAYMWLDAELTSGSGRSQCERKLGQFFKHQIESDTSLVYGAGFRAGHQAVLKYGLPATLKHIHLTGNFPY

SEQ ID NO: 13 - protein, 482 aa, Vitis vinifera
MGWLNKIFKGSSHKISEGNYHGRYQGDTVQNEPSCSGDVWAETENEDIDRAIALSLSEEEQKGKKVIDELDNEFQLEEDEQLARAIQESLNIESPPQHGNGNGNGNIYQPIPFPYSTGFRICAGCNTEIGHGRFLSCMGAVWHPECFRCHGCGYPISDYEYSMNGNYPYHKSCYKEHYHPKCDVCKHFIPTNPAGLIEYRAHPFWVQKYCPSHEHDRTPRCCSCERMEPRDTRYVALNDGRKLCLECLDSAIMDTNECQPLYLDIQEFYEGLNMKVQQQVPLLLVERQALNEAMEGEKSGHHHMPETRGLCLSEEQTVSTILRRPKIGTGNRVMNMITEPCKLTRRCDVTAVLILYGLPRLLTGSILAHEMMHAWLRLNGYRTLAQDVEEGICQVLAYMWLDAELTSGSGSNVPSTSSASTSSKKGAGSQCERKLGQFFKHQIESDTSLVYGAGFRAGHQAVLKYGLPATLKHIHLTGNFPY

SEQ ID NO: 14 - protein, 486 aa, Solanum lycopersicum
MGWLNKIFRGSSHKISEGQYDWRCEGHTEEDDPSTAEDSWSEIEEIDRAIAISLSEEEQKGKIVIDSESQLKEDEQLARALQESLNVESPPQHVSRNDHGGGNVYGNGNFYHPVPFPYSASFRVCAGCSTEIGHGRFLSCMGAVWHPECFRCHACNQPISDYEFSMSGNYPYHKTCYKEHYHPKCDVCKHFIPTNAAGLIEYRAHPFWSQKYCPFHEHDGTPRCCSCERMEPRDTRYIALDDGRKLCLECLDSAIMDTSQCQPLYYDIQEFYEGLNMKVEQKVPLLLVERQALNEAMDGERHGYHHMPETRGLCLSEEQTISTIQRRPRIGAGNRVMDMRTEPYKLTRRCEVTAILILYGLPRLLTGSILAHEMMHAWLRLRGYRTLSQDVEEGICQVLAHMWLETQIASISSSNGGASTSSGMSSSKQGIRSPFERKLGDFFKHQIESDTSPIYGNGFRAGNQAVLKYGLERTLDHIRMTGTFPY

SEQ ID NO: 15 - protein, 878 aa, Oryza sativa
MGDRPDMGAGVALRFSHNDWTLEEDSKALHFLQPDLVLFTGDYGNENVQLVKSISDLQLPKAAILGNHDCWHTYQFSEKKVDRVQLQLESLGEQHVGYKCLDFPTIKLSVVGGRPFSCGGNRIFRPKLLSKWYGVNDMAESAKRIYDAATNAPKEHAVILLAHNGPTGLGSRMEDICGRDWVAGGGDHGDPDLEQAISDLQRETGVSIPLVVFGHMHKSLAYGRGLRKMIAFGANRTIYLNGAVVPRVNHAQSSRQPAISTSEKTGLEGLTGLMVPTSRAFTIVDLFEGAVEKISEVWVTVGDARTELEQELVLYKQPHKSVPSNIAIWSTMGWLTKFFRGSTHKISEGQYHSKPAEETIWNGPSNSAVVTMVYPLESTFGQLDLLLLATDLRQLVIDDVDCCKLRQQAQPVLHLMYSQLQLLQTSHAHQHGDVPSEFDNEDIARAISLSLLEEEQRKAKAIEKDMHLEEDEQLARAIQESLNVESPPRARENGNANGGNMYQPLPFMFSSGFRTCAGCHSEIGHGRFLSCMGAVWHPECFRCHACNQPIYDYEFSMSGNHPYHKTCYKERFHPKCDVCKQFIPTNMNGLIEYRAHPFWLQKYCPSHEVDGTPRCCSCERMEPRESRYVLLDDGRKLCLECLDSAVMDTSECQPLYLEIQEFYEGLNMKVEQQVPLLLVERQALNEAMEGEKTGHHHLPETRGLCLSEEQTVSTILRRPRMAGNKVMEMITEPYRLTRRCEVTAILILYGLPRLLTGSILAHEMMHAWLRLKGYRTLSPDVEEGICQVLAHMWIESEIIAGSGSNGASTSSSSSASTSSKKGGRSQFERKLGDFFKHQIESDTSMAYGDGFRAGNRAVLQYGLKRTLEHIRLTGTFPF

SEQ ID NO: 16 - protein, 486 aa, Oryza sativa
MGWLTKFFRGSTHKISEGQYHSKPAEETIWNGPSNSAVVTDVPSEFDNEDIARAISLSLLEEEQRKAKAIEKDMHLEEDEQLARAIQESLNVESPPRARENGNANGGNMYQPLPFMFSSGFRTCAGCHSEIGHGRFLSCMGAVWHPECFRCHACNQPIYDYEFSMSGNHPYHKTCYKERFHPKCDVCKQFIPTNMNGLIEYRAHPFWLQKYCPSHEVDGTPRCCSCERMEPRESRYVLLDDGRKLCLECLDSAVMDTSECQPLYLEIQEFYEGLNMKVEQQVPLLLVERQALNEAMEGEKTGHHHLPETRGLCLSEEQTVSTILRRPRMAGNKVMEMITEPYRLTRRCEVTAILILYGLPRLLTGSILAHEMMHAWLRLKGYRTLSPDVEEGICQVLAHMWIESEIIAGSGSNGASTSSSSSASTSSKKGGRSQFERKLGDFFKHQIESDTSMAYGDGFRAGNRAVLQYGLKRTLEHIRLTGTFPF

SEQ ID NO: 17 - protein, 512 aa, Brachypodium distachyon
MGWLTKIFRGSTYKISEGQRQSRPAEEAVWNEPSSSTVVTDVLSEFDNEDIDRAIALSLSEEQRKSKGTGKDLHLDEDEQLARAIHESLNVESPPCARDNGSPPHARDNSSPPHARENSSHPRARENGIANGGNSIQHSPFMFSSGFRTCAGCHSEIGHGRFLSCMGAVWHPECFCCHACSQPIYDYEFSMSGNHPYHKTCYKERFHPKCDVCKQFIPTNMNGLIEYRAHPFWLQKYCPSHEVDGTPRCCSCERMEPRESRYVLLDDGRKLCLECLDSAVMDTTECQPLYLEIQEFYEGLNMKVEQQVPLLLVERQALNEAMEGEKTGHHHLPETRGLCLSEEQTVSTILRRPRMTGNKIMEMITEPYRLTRRCEVTAILILYGLPRLLTGSILAHEMMHAWLRLKGYRTLSPEIEEGICQVLAHMWIESEIMAGSSSNAASTSSSSSSSISSKKGGRSQFERKLGDFFKHQIESDTSVAYGNGFRSGNQAVLQYGLKRTLEHIWLTGTWPF

SEQ ID NO: 18 - protein, 491 aa, Brachypodium distachyon
MGWLTKFFRGSTHNISEGQDQSKPAEETVWNEPSSSTAVNYALSEFDNEDIDRAIALSLSEEEQRKSKGTGKDQHLDEDEQLARAIQESLNVESPPRAREKSSHPRARENGSANGGNSYQLPLMFSSGFRTCAGCHSEIGHGRFLSCMGAVWHPECFCCHGCSQPIYDYEFSMSGNHPYHKTCYKERFHPKCDVCQQFIPTNTNGLIEYRAHPFWLQKYCPSHEVDGTPRCCSCERMEPRESRYVLLDDGRKLCLECLDSAVMDTTECQPLYLEIQEFYEGLNMKVEQQVPLLLVERQALNEAMEGEKTGHHHLPETRGLCLSEEQTVSTILRRPRMAGNKIMEMRTEPYRLTRRCEVTAILILYGLPRLLTGSILAHEMMHAWLRLKGYRTLSPDIEEGICQVLAHMWIESEITAGSGSNAASTSSSSTSSKKGGRSQFERKLGDFFKHQIESDTSVAYGDGFRAGNQAVLQYGLKRTLEHIRLTGTLPF

SEQ ID NO: 19 - protein, 486 aa, Sorghum bicolor
MGWLTKFFRGSTHNISEGQYHSRPAEDTAWNEPSSSPVVTDIFSEFNNEDIDRAIALSLSEEEQRKAKTIDKDMHLEEDEQLARAIQESLNVESPPPSRENGSANGGNAYHPLPFMFSSGFRACAGCHREIGHGRFLSCMGAVWHPECFRCHACSQPIYDYEFSMSGNHPYHKTCYKEQFHPKCDVCKQFIPTNMNGLIEYRAHPFWLQKYCPSHEVDGTPRCCSCERMEPRESRYVLLDDGRKLCLECLDSAVMDTNECQPLYLEIQEFYEGLNMKVEQQVPLLLVERQALNEAMEGEKAGHHHLPETRGLCLSEEQTVSTILRRPRMAGNKIMGMITEPYRLTRRCEVTAILILYGLPRLLTGSILAHEMMHAWLRLKGYRTLSPDVEEGICQVLAHLWIESEIMAGSGSGAASSSSGSSSSMSSKKAGRSQFEHKLGDFFKHQIETDTSMAYGEGFRAGNRAVLQYGLKRTLEHIRLTGTFPF

SEQ ID NO: 20 - protein, 508 aa, Zea mays
MGWLTKFFRGSTHNISEEQYHSRPAEDTAWNEPSSSPVVTDILSEFNNEDIDRAIALSLSEEEQRKEKAIDKDMHLEEDEQLARAIQESLNVESPPRRNGSANGGTMYHPPRETGNAYQPPRENGSANGGNAYHPLPFMFSSGFRACAGCHREIGHGRFLSCMGAVWHPECFRCHACSQPIYDYEFSMSGNHPYHKTCYKEQFHPKCDVCKQFIPTNMNGLIEYRAHPFWVQKYCPSHEMDGTPRCCSCERMEPRESKYVLLDDGRKLCLECLDSAVMDTNDCQPLYLEIQEFYEGLNMKVEQQVPLLLVERQALNEAMEGEKAGHHHLPETRGLCLSEEQTVSTILRPRMAGNKIMGMITEPYRLTRRCEVTAILILYGLPRLLTGSILAHEMMHAWLRLKGYRTLSPDVEEGICQVLAHMWIESEIMAGSGSSAASSSSGSSSSTSSKKGGRSQFEHRLGDFFKHQIETDTSMAYGDGFRTGNRAVLHYGLKRTLEHIRLTGTFPF

SEQ ID NO: 21 - protein, 553 aa, Arabidopsis thaliana
MGWLTKILKGSSHKFSDGQCNGRYREDRNLEGPRYSAEGSDFDKEEIECAIALSLSEQEHVIPQDDKGKKIIEYKSETEEDDDDDEDEDEEYMRAQLEAAEEEERRVAQAQIEEEEKRRAEAQLEETEKLLAKARLEEEEMRRSKAQLEEDELLAKALQESMNVGSPPRYDPGNILQPYPFLIPSSHRICVGCQAEIGHGRFLSCMGGVWHPECFCCNACDKPIIDYEFSMSGNRPYHKLCYKEQHHPKCDVCHNFIPTNPAGLIEYRAHPFWMQKYCPSHERDGTPRCCSCERMEPKDTKYLILDDGRKLCLECLDSAIMDTHECQPLYLEIREFYEGLHMKVEQQIPMLLVERSALNEAMEGEKHGHHHLPETRGLCLSEEQTVTTVLRRPRIGAGYKLIDMITEPCRLIRRCEVTAILILYGLPRLLTGSILAHEMMHAWLRLNGYPNLRPEVEEGICQVLAHMWLESETYAGSTLVDIASSSSSAVVSASSKKGERSDFEKKLGEFFKHQIESDSSSAYGDGFRQGNQAVLKHGLRRTLDHIRLTGTFP

SEQ ID NO: 22 - protein, 528 aa, Arabidopsis thaliana
MDSSSSSSSSSPSSSYGVARVSHISNPCIFGEVGSSSSSTYRDKKWKLMKWVSKLFKSGSNGGGSGAHTNHHPPQFQEDENMVFPLPPSSLDDRSRGARDKEELDRSISLSLADNTKRPHGYGWSMDNNRDFPRPFHGGLNPSSFIPPYEPSYQYRRRQRICGGCNSDIGSGNYLGCMGTFFHPECFRCHSCGYAITEHEFSLSGTKPYHKLCFKELTHPKCEVCHHFIPTNDAGLIEYRCHPFWNQKYCPSHEYDKTARCCSCERLESWDVRYYTLEDGRSLCLECMETAITDTGECQPLYHAIRDYYEGMYMKLDQQIPMLLVQREALNDAIVGEKNGYHHMPETRGLCLSEEQTVTSVLRRPRLGAHRLVGMRTQPQRLTRKCEVTAILVLYGLPRLLTGAILAHELMHGWLRLNGFRNLNPEVEEGICQVLSYMWLESEVLSDPSTRNLPSTSSVATSSSSSFSNKKGGKSNVEKKLGEFFKHQIAHDASPAYGGGFRAANAAACKYGLRRTLDHIRLTGTFPL

SEQ ID NO: 23 - protein, 1613 aa, Arabidopsis thaliana
MEPPAARVTPSIKADCSHSVNIICEETVLHSLVSHLSAALRREGISVFVDACGLQETKFFSIKQNQPLTDGARVLVVVISDEVEFYDPWFPKFLKVIQGWQNNGHVVVPVFYGVDSLTRVYGWANSWLEAEKLTSHQSKILSNNVLTDSELVEEIVRDVYGKLYPAERVGIYARLLEIEKLLYKQHRDIRSIGIWGMPGIGKTTLAKAVFNHMSTDYDASCFIENFDEAFHKEGLHRLLKERIGKILKDEFDIESSYIMRPTLHRDKLYDKRILVVLDDVRDSLAAESFLKRLDWFGSGSLIIITSVDKQVFAFCQINQIYTVQGLNVHEALQLFSQSVFGINEPEQNDRKLSMKVIDYVNGNPLALSIYGRELMGKKSEMETAFFELKHCPPLKIQDVLKNAYSALSDNEKNIVLDIAFFFKGETVNYVMQLLEESHYFPRLAIDVLVDKCVLTISENTVQMNNLIQDTCQEIFNGEIETCTRMWEPSRIRYLLEYDELEGSGETKAMPKSGLVAEHIESIFLDTSNVKFDVKHDAFKNMFNLKFLKIYNSCSKYISGLNFPKGLDSLPYELRLLHWENYPLQSLPQDFDFGHLVKLSMPYSQLHKLGTRVKDLVMLKRLILSHSLQLVECDILIYAQNIELIDLQGCTGLQRFPDTSQLQNLRVVNLSGCTEIKCFSGVPPNIEELHLQGTRIREIPIFNATHPPKVKLDRKKLWNLLENFSDVEHIDLECVTNLATVTSNNHVMGKLVCLNMKYCSNLRGLPDMVSLESLKVLYLSGCSELEKIMGFPRNLKKLYVGGTAIRELPQLPNSLEFLNAHGCKHLKSINLDFEQLPRHFIFSNCYRFSSQVIAEFVEKGLVASLARAKQEELIKAPEVIICIPMDTRQRSSFRLQAGRNAMTDLVPWMQKPISGFSMSVVVSFQDDYHNDVGLRIRCVGTWKTWNNQPDRIVERFFQCWAPTEAPKVVADHIFVLYDTKMHPSDSEENHISMWAHEVKFEFHTVSGENNPLGASCKVTECGVEVITAATGDTSVSGIIRESETITIIEKEDTIIDEEDTPLLSRKPEETNRSRSSSELQKLSSTSSKVRSKGNVFWKWLGCFPLQPKNLRSRSRRTTALEEALEEALKEREKLEDTRELQIALIESKKIKKIKQADERDQIKHADEREQRKHSKDHEEEEIESNEKEERRHSKDYVIEELVLKGKGKRKQLDDDKADEKEQIKHSKDHVEEEVNPPLSKCKDCKSAIEDGISINAYGSVWHPQCFCCLRCREPIAMNEISDLRGMYHKPCYKELRHPNCYVCEKKIPRTAEGLKYHEHPFWMETYCPSHDGDGTPKCCSCERLEHCGTQYVMLADFRWLCRECMDSAIMDSDECQPLHFEIREFFEGLHMKIEEEFPVYLVEKNALNKAEKEEKIDKQGDQCLMVVRGICLSEEQIVTSVSQGVRRMLNKQILDTVTESQRVVRKCEVTAILILYGLPRLLTGYILAHEMMHAYLRLNGYRNLNMVLEEGLCQVLGYMWLECQTYVFDTATIASSSSSSRTPLSTTTSKKVDPSDFEKRLVNFCKHQIETDESPFFGDGFRKVNKMMASNNHSLKDTLKEIISISKTPQYSKL

SEQ ID NO: 24 - protein, 450 aa, Arabidopsis thaliana
MVRRKRQEEDEKIEIERVKEESLKLAKQAEEKRRLEESKEQGKRIQVDDDQLAKTTSKDKGQINHSKDVVEEDVNPPPSIDGKSEIGDGTSVNPRCLCCFHCHRPFVMHEILKKGKFHIDCYKEYYRNRNCYVCQQKIPVNAEGIRKFSEHPFWKEKYCPIHDEDGTAKCCSCERLEPRGTNYVMLGDFRWLCIECMGSAVMDTNEVQPLHFEIREFFEGLFLKVDKEFALLLVEKQALNKAEEEEKIDYHRAAVTRGLCMSEEQIVPSIIKGPRMGPDNQLITDIVTESQRVSGFEVTGILIIYGLPRLLTGYILAHEMMHAWLRLNGYKNLKLELEEGLCQALGLRWLESQTFASTDAAAAAAVASSSSFSSSTAPPAAITSKKSDDWSIFEKKLVEFCMNQIKEDDSPVYGLGFKQVYEMMVSNNYNIKDTLKDIVSASNATPDSTV

SEQ ID NO: 25 - protein, 702 aa, Arabidopsis thaliana
MPISDVASLVGGAALGAPLSEIFKLVIEEAKKVKDFKPLSQDLASTMERLVPIFNEIDMMQQGSNRGTSELKVLTETMERAGEMVHKCSRIQWYSIAKKALYTREIKAINQDFLKFCQIELQLIQHRNQLQYMRSMGMASVSTKADLLSDIGNEFSKLCLVAQPEVVTKFWLKRPLMELKKMLFEDGVVTVVVSAPYALGKTTLVTKLCHDADVKEKFKQIFFISVSKFPNVRLIGHKLLEHIGCKANEYENDLDAMLYIQQLLKQLGRNGSILLVLDDVWAEEESLLQKFLIQLPDYKILVTSRFEFTSFGPTFHLKPLIDDEVECRDEIEENEKLPEVNPPLSMCGGCNSAVKHEESVNILGVLWHPGCFCCRSCDKPIAIHELENHVSNSRGKFHKSCYERYCYVCKEKKMKTYNIHPFWEERYCPVHEADGTPKCCSCERLEPRGTKYGKLSDGRWLCLECGKSAMDSDECQPLYFDMRDFFESLNMKIEKEFPLILVRKELLNKKEEKIDNHYEVLIRAYCMSEQKIMTYVSEEPRTGQNKQLIDMDTEPQGVVHECKVTAILILYGLPRLLTGYILAHEMMHAWLRLNGHMNLNNILEEGICQVLGHLWLESQTYATADTTADAASASSSSSRTPPAASASKKGEWSDFDKKLVEFCKNQIETDESPVYGLGFRTVNEMVTNSSLQETLKEILRRR

SEQ ID NO: 26 - protein, 644 aa, Arabidopsis thaliana
MASDYYSSDDEGFGEKVGLIGEKDRFEAETIHVIEVSQHEADIQKAKQRSLATHEAEKLDLATHEAEQLDLAIQEFSRQEEEEERRRTRELENDAQIANVLQHEERERLINKKTALEDEEDELLARTLEESLKENNRRKMFEEQVNKDEQLALIVQESLNMEEYPIRLEEYKSISRRAPLDVDEQFAKAVKESLKNKGKGKQFEDEQVKKDEQLALIVQESLNMVESPPRLEENNNISTRAPVDEDEQLAKAVEESLKGKGQIKQSKDEVEGDGMLLELNPPPSLCGGCNFAVEHGGSVNILGVLWHPGCFCCRACHKPIAIHDIENHVSNSRGKFHKSCYERYCYVCKEKKMKTYNNHPFWEERYCPVHEADGTPKCCSCERLEPRESNYVMLADGRWLCLECMNSAVMDSDECQPLHFDMRDFFEGLNMKIEKEFPFLLVEKQALNKAEKEEKIDYQYEVVTRGICLSEEQIVDSVSQRPVRGPNNKLVGMATESQKVTRECEVTAILILYGLPRLLTGYILAHEMMHAYLRLNGHRNLNNILEEGICQVLGHLWLDSQTYATADATADASSSASSSSRTPPAASASKKGEWSDFDKKLVEFCKNQIETDDSPVYGLGFRTVNEMVTNSSLQETLKEILRQR

SEQ ID NO: 27 - protein, 587 aa, Arabidopsis thaliana
MWCLSCFKPSTKHDPSEDRFEEETNIVTGISLYEDVILRQRRSEADQIEWAIQDSFNPQETSRCRQREEDDQIARGLQYVEETELDKSVVDEEDQQLSKIVEESLKEKGKSKQFEDDQVENDEQQALMVQESLYMVELSAQLEEDKNISTIPPLNEDAQLQKVIWESAKGKGQIEHFKDPVEEDGNLPRVDLNVNHPHSICDGCKSAIEYGRSVHALGVNWHPECFCCRYCDKPIAMHEFSNTKGRCHITCYERSHPNCHVCKKKFPGRKYKEHPFWKEKYCPFHEVDGTPKCCSCERLEPWGTKYVMLADNRWLCVKCMECAVMDTYECQPLHFEIREFFGSLNMKVEKEFPLLLVEKEALKKAEAQEKIDNQHGVVTRGICLSEGQIVNSVFKKPTMGPNGELVSLGTEPQKVVGGCEVTAILILYGLPRLLTGYILAHEMMHAWLRLNGTTSTQFVFANQYGESSQLKVLFGLITGYRNLKLELEEGICQVLGHMWLESQTYSSSAAASSASSSSRTPAANASKKGAQSDYEKKLVEFCKDQIETDDSPVYGVGFRKVNQMVSDSSLHKILKSIQHWTKPDSNL

SEQ ID NO: 28 - protein, 73 aa, Artificial sequence
  Synthetic sequence: LIM-like domain
  VARIANT (2)..(3): Xaa is any amino acid
  VARIANT (5)..(27): Xaa at positions 5 to 27 is any amino acid and up to seven of them may be absent; represents a range of 16 - 23 amino acids.
  VARIANT (29)..(35): Xaa is any amino acid
  VARIANT (37)..(38): Xaa is any amino acid
  VARIANT (40)..(46): Xaa is any amino acid
  VARIANT (48)..(49): Xaa is any amino acid
  VARIANT (51)..(69): Xaa is any amino acid
  VARIANT (71)..(72): Xaa is any amino acid
CXXCXXXXXXXXXXXXXXXXXXXXXXXHXXXXXXXCXXHXXXXXXXCXXCXXXXXXXXXXXXXXXXXXXCXXC

SEQ ID NO: 29 - protein, 73 aa, Artificial sequence
  Synthetic sequence: LIM-like domain
  VARIANT (2)..(2): Xaa is any amino acid
  VARIANT (5)..(27): Xaa at positions 5 to 27 is any amino acid and up to seven of them may be absent; represents a range of 16 - 23 amino acids.
  VARIANT (32)..(34): Xaa is any amino acid
  VARIANT (38)..(38): Xaa is any amino acid
  VARIANT (40)..(46): Xaa is any amino acid
  VARIANT (53)..(53): Xaa is any amino acid
  VARIANT (55)..(59): Xaa is any amino acid
  VARIANT (61)..(62): Xaa is any amino acid
  VARIANT (64)..(64): Xaa is any amino acid
  VARIANT (66)..(66): Xaa is any amino acid
  VARIANT (68)..(68): Xaa is any amino acid
  VARIANT (71)..(72): Xaa is any amino acid
CXVCXXXXXXXXXXXXXXXXXXXXXXXHPFWXXXYCPXHXXXXXXXCCSCERXEXXXXXYXXLXDXRXLCXXC

SEQ ID NO: 30 - protein, 66 aa, Artificial sequence
  Synthetic sequence: LIM-like domain
  VARIANT (2)..(2): Xaa is Asp, Glu, Tyr or His
  VARIANT (5)..(6): Xaa is any amino acid
  VARIANT (7)..(7): Xaa is Phe or Lys
  VARIANT (8)..(8): Xaa is Ile, Lys or Phe
  VARIANT (9)..(9): May be present or absent. If present, Xaa is Pro or Ser
  VARIANT (10)..(10): May be present or absent. If present, Xaa is Thr, Arg or Val
  VARIANT (11)..(11): May be present or absent. If present, Xaa is Asn or Thr
  VARIANT (12)..(13): Xaa is any amino acid
  VARIANT (14)..(14): May be present or absent. If present, Xaa is Gly
  VARIANT (15)..(15): Xaa is Leu, Ile, Met or Gly
  VARIANT (16)..(16): Xaa is Arg, Lys or Ile
  VARIANT (17)..(17): Xaa is Glu, Gly, Lys or Thr
  VARIANT (18)..(18): Xaa is Tyr or Phe
  VARIANT (19)..(19): Xaa is Arg, His, Ser, Asn or Lys
  VARIANT (20)..(20): Xaa is Ala, Cys, Glu, Ile or Asn
  VARIANT (25): Xaa is any amino acid
  VARIANT (26)..(26): Xaa is Gln or Glu
  VARIANT (27)..(27): Xaa is Lys, Thr or Arg
  VARIANT (31)..(31): Xaa is Phe, Val, Ile, Ser or Thr
  VARIANT (33)..(33): Xaa is Glu or Asp
  VARIANT (34)..(34): Xaa is any amino acid
  VARIANT (36)..(36): Xaa is Gly, Lys, Arg, Ser or Ala
  VARIANT (38)..(38): Xaa is Pro, Thr or Ala
  VARIANT (39)..(39): Xaa is Arg or Lys
  VARIANT (46)..(46): Xaa is Met or Leu
  VARIANT (48)..(48): Xaa is Pro, Ser or His
  VARIANT (49)..(52): Xaa is any amino acid
  VARIANT (54)..(55): Xaa is any amino acid
  VARIANT (57)..(57): Xaa is any amino acid
  VARIANT (59)..(59): Xaa is Gly, Phe or Asn
  VARIANT (61)..(61): Xaa is Arg, Lys, Ser or Trp
  VARIANT (64)..(64): Xaa is Leu, Arg or Val
  VARIANT (65)..(65): Xaa is Glu or Lys
CXVCXXXXXXXXXXXXXXXXHPFWXXXYCPXHXXDXTXXCCSCERXEXXXXXYXXLXDXRXLCXXC

SEQ ID NO: 31 - protein, 66 aa, Arabidopsis thaliana
CDVCSHFIPTNHAGLIEYRAHPFWVQKYCPSHEHDATPRCCSCERMEPRNTRYVELNDGRKLCLEC

SEQ ID NO: 32 - protein, 5 aa, Artificial sequence
  Synthetic sequence: Metallopeptidase active site motif
HEMMH

SEQ ID NO: 33 - protein, 19 aa, Artificial sequence
  Synthetic sequence: Carboxyl terminal region motif
  VARIANT (3)..(10): Xaa is any amino acid
  VARIANT (12)..(15): Xaa is any amino acid
EKXXXXXXXXRXXXXSEEQ

SEQ ID NO: 34 - protein, 18 aa, Artificial sequence
  Synthetic sequence: Carboxyl terminal region motif
  VARIANT (3)..(10): Xaa is any amino acid
  VARIANT (12)..(15): Xaa is any amino acid
EKXXXXXXXXRXXXXSEQ

SEQ ID NO: 35 - protein, 21 aa, Artificial sequence
  Synthetic sequence: UIM1 domain
  VARIANT (1)..(1): Xaa is a polar amino acid residue, for example Cys, Asp, Glu, His, Lys, Asn, Gln, Arg, Ser or Thr
  VARIANT (2)..(4): Xaa is any amino acid
  VARIANT (5)..(5): Xaa is a polar amino acid residue, for example Cys, Asp, Glu, His, Lys, Asn, Gln, Arg, Ser or Thr
  VARIANT (7)..(7): Xaa is a polar amino acid residue, for example Cys, Asp, Glu, His, Lys, Asn, Gln, Arg, Ser or Thr
  VARIANT (8)..(8): Xaa is a big amino acid residue, for example Glu, Phe, His, Ile, Lys, Met, Gln, Arg, Trp or Tyr
  VARIANT (10)..(10): Xaa is an aliphatic amino acid residue, for example Ile, Leu or Val
  VARIANT (11)..(11): Xaa is a polar amino acid residue, for example Cys, Asp, Glu, His, Lys, Asn, Gln, Arg, Ser or Thr
  VARIANT (12)..(12): Xaa is a big amino acid residue, for example Glu, Phe, His, Ile, Lys, Met, Gln, Arg, Trp or Tyr
  VARIANT (13)..(13): May be present or absent. If present, Xaa is any amino acid.
  VARIANT (15)..(15): Xaa is a big amino acid residue, for example Glu, Phe, His, Ile, Lys, Met, Gln, Arg, Trp or Tyr
  VARIANT (16)..(16): Xaa is a polar amino acid residue, for example Cys, Asp, Glu, His, Lys, Asn, Gln, Arg, Ser or Thr
  VARIANT (17)..(17): Xaa is any amino acid
  VARIANT (18)..(18): May be present or absent. If present, Xaa is any amino acid.
  VARIANT (19)..(21): Xaa is a polar amino acid residue, for example Cys, Asp, Glu, His, Lys, Asn, Gln, Arg, Ser or Thr
XXXXXLXXAXXXXSXXXXXXX

SEQ ID NO: 36 - protein, 21 aa, Artificial sequence
  Synthetic sequence: UIM2 domain
  VARIANT (1)..(1): Xaa is a polar amino acid residue, for example Cys, Asp, Glu, His, Lys, Asn, Gln, Arg, Ser or Thr
  VARIANT (2)..(4): Xaa is any amino acid
  VARIANT (5)..(5): Xaa is a polar amino acid residue, for example Cys, Asp, Glu, His, Lys, Asn, Gln, Arg, Ser or Thr
  VARIANT (7)..(7): Xaa is a polar amino acid residue, for example Cys, Asp, Glu, His, Lys, Asn, Gln, Arg, Ser or Thr
  VARIANT (8)..(8): Xaa is a big amino acid residue, for example Glu, Phe, His, Ile, Lys, Met, Gln, Arg, Trp or Tyr
  VARIANT (10)..(10): Xaa is an aliphatic amino acid residue, for example Ile, Leu or Val
  VARIANT (11)..(11): Xaa is a polar amino acid residue, for example Cys, Asp, Glu, His, Lys, Asn, Gln, Arg, Ser or Thr
  VARIANT (12)..(12): Xaa is a big amino acid residue, for example Glu, Phe, His, Ile, Lys, Met, Gln, Arg, Trp or Tyr
  VARIANT (13)..(13): May be present or absent. If present, Xaa is any amino acid.
  VARIANT (15)..(15): Xaa is a big amino acid residue, for example Glu, Phe, His, Ile, Lys, Met, Gln, Arg, Trp or Tyr
  VARIANT (16)..(16): Xaa is a polar amino acid residue, for example Cys, Asp, Glu, His, Lys, Asn, Gln, Arg, Ser or Thr
  VARIANT (17)..(17): Xaa is any amino acid
  VARIANT (18)..(18): Xaa is a small amino acid residue, for example Ala, Cys, Asp, Gly, Asn, Pro, Ser, Thr or Val
  VARIANT (19)..(21): Xaa is a polar amino acid residue, for example Cys, Asp, Glu, His, Lys, Asn, Gln, Arg, Ser or Thr
XXXXXLXXAXXXXSXXXXXXX

SEQ ID NO: 37 - protein, 43 aa, Artificial sequence
  Synthetic sequence: Plant EOD domain
  VARIANT (1)..(1): Xaa is Glu or Lys
  VARIANT (8)..(8): Xaa is Leu or Met
  VARIANT (9)..(9): Xaa is Lys, Arg, Gly, Thr or Glu
  VARIANT (11)..(11): Xaa is Lys or Arg
  VARIANT (12)..(12): Xaa is Arg or Ile
  VARIANT (13)..(13): Xaa is Gly or Lys
  VARIANT (14)..(14): Xaa is Asp, Asn or Glu
  VARIANT (15)..(15): Xaa is Arg, Gln, Lys or Leu
  VARIANT (17)..(17): Xaa is Ile, Met or Val
  VARIANT (18)..(18): Xaa is Lys, Asn, Thr or Ala
  VARIANT (20)..(20): Xaa is Leu or Pro
  VARIANT (22)..(22): Xaa is Lys or Ser
  VARIANT (24)..(24): Xaa is Val or Ala
  VARIANT (27)..(27): Xaa is Ser, Thr, Gly or Ala
  VARIANT (28)..(28): Xaa is Glu, Gln, Asp, Ser or Gly
  VARIANT (30)..(30): Xaa is Ile, Gly, Thr or Val
  VARIANT (31)..(31): Xaa is Ser or Thr
  VARIANT (32)..(32): Xaa is Lys or Arg
  VARIANT (35)..(35): Xaa is Gly, Thr or Ser
  VARIANT (39)..(39): Xaa is Val, Ile, Ala or Lys
  VARIANT (42)..(42): Xaa is Val or Ile
XRCVICQXXYXXXXXQXXLXCXHXYHXXCXXXWLXINKXCPXC

SEQ ID NO: 38 - protein, 203 aa, Populus trichocarpa
MEVHYMNTDFPYTTTESFMDFFEGLTHAPVNYAHNGPMHDQDNAYWSMNMNAYKFGFSGLGSTSYYSPYEVNDNLPRMDVSRMAWEYPSVVIKALWQDDVDPDTMTYEELVDLGETVGTQSKGLSPELISLLPTSKCKFGSFFSRKRSGERCVICQMKYKRGDKQIKLLCKHAYHSECITKWLGINKVCPVCNDEVFGEESRN

SEQ ID NO: 39 - protein, 240 aa, Ricinus communis
MEVHYINTGFPYTVTESFLDFFEGLSHVPVHYAHTGQVLDQVQENAYWSMNMNAYKYGFSGPGSTYYDPYEVNDNLPRMDVSRSTWEYPSVVNMEEATTTDTQSEGDAVVGVHASPEECIPNHTSGDSPQGVWQDDVDPDNMTYEELLDLGETVGTQSRGLSQELISLLPTSKCKFRSFFLRKKAGERCVICQMRYKRGDKQMKLPCKHVYHSECISKWLGINKVCPVCNNEVFGEDSRH

SEQ ID NO: 40 - protein, 245 aa, Prunus persica
MNGNGQMDVHYIDTDFPYTPTESFMDFFGGVTHVPMNYGHAMPMHDQETAYWSMNMHSYKFGPSGPGSNSYYGNYYEVNDHLPRMDVSRRTWEHPSVMNSEEPANIDSHPEEEDAVAEAAPEECIQNQQNTNTSQVVWQEDIDPDNMTYEELLDLGEAVGTQSRGLSDELISLLPTSKYKCGSFFSRKKSGERCVICQMRYKRGDRQINLPCKHVYHSECISKWLGINKVCPVCNLEVSGEESRH

SEQ ID NO: 41 - protein, 242 aa, Theobroma cacao
MNGNRQMEVHYIDTGFPYTATESFMDFFEGLTHVPVNYTHTVPMQDQENIYWSMSMNAYKFGFSGPESTFYSPYEVSDHLPRMDVSRRTWDYPSTLNSEEPATIDMQPGGEAVVGIHAIPEECITNHQSNSNSQVVWQDNIDPDNMTYEELLDLGETIGSQSRGLSQELIDLLPTSKCKFGSFFSTKRERCVICQMRYKRGEQQMKLPCKHVYHSQCITKWLSINKICPVCNNEVFGEESRH

SEQ ID NO: 42 - protein, 247 aa, Vitis vinifera
MNGNRQMEVHYINTGFPYTITESFMDFFEGLGHVPVNYAQAEAMHNQSIQENFYWTMNMNSYKFGFSGPGSTYYGPYDVNEHVPGIEVSRRPWEYPSSMIVEEPTTIETQPTGNEVMNVHAIPEECSPNHYSATSSQAIWQDNVDPDNMTYEELLDLGEAVGTQSRGLSQEHINLLPTCRYKSGRLFSRKRSAERCVICQMGYKRGDRQIKLPCKHVYHTDCGTKWLTINKVCPVCNIEVFGEESRH

SEQ ID NO: 43 - protein, 247 aa, Glycine max
MNDGRQMGVHYVDAGFPYAVNDNFVDFFQGFTHVPVNYAFAGSIPDQESVYWSMNMNPYKFGLSGPGSTSYYSSYEVNGHLPRMEIDRAEWEYPSTITTVEEPATTDSPPRRDGVTSMQTIPEECSPNHHESNSSSQVIWQDNIYPDDMTYEELLDLGEAVGTQSRGLSQELIDMLPTSKYKFGSLFKRKNSGKRCVICQMTYRRGDQQMKLPCSHVYHGECITKWLSINKKCPVCNTEVFGEESTH

SEQ ID NO: 44 - protein, 247 aa, Glycine max
MNDGRQMGVNYVDAGFPYAVNENFVDFFQGFTPVPVNYAFAGSIPDQESVYWSMNMNPYKFGLSGPGSTSYYSSYEVNGHLPRMEIDRAEWEYPSTITTVEEPATTDSPPRRDGVTNMQTIPEECSPNHHESNSSSQVIWQDNIDPDNMTYEELLDLGEAVGTQSRGLSQELIDMLPTSKYKFGNLFKRKNSGKRCVICQMTYRRGDQQMKLPCSHVYHGECITKWLSINKKCPVCNTEVFGEESTH

SEQ ID NO: 45 - protein, 248 aa, Arabidopsis thaliana
MNGDNRPVEDAHYTETGFPYAATGSYMDFYGGAAQGPLNYDHAATMHPQDNLYWTMNTNAYKFGFSGSDNASFYGSYDMNDHLSRMSIGRTNWDYHPMVNVADDPENTVARSVQIGDTDEHSEAEECIANEHDPDSPQVSWQDDIDPDTMTYEELVELGEAVGTESRGLSQELIETLPTKKYKFGSIFSRKRAGERCVICQLKYKIGERQMNLPCKHVYHSECISKWLSINKVCPVCNSEVFGEPSIH

SEQ ID NO: 46 - protein, 243 aa, Capsella rubella
MNGDRPVEDAHYTEAEFPYAASGSYIDFYGGAPQGPLNYAHAGTMDNLYWTMNTNAYKFGFSGSDNPSFYNSYDMTDHLSRMSIGRTNWEYHPMVNVDDPDITLARSVQIGDSDEHSEAEDCIANEHDPDSPQVSWQDDIDPDTMTYEELVELGEAVGTESRGLSQELIETLPTRKFKFGSIFSRKRAGERCVICQLKYKIGERQMNLPCKHVYHSECISKWLSINKVCPVCNTEVFGDPSIH

SEQ ID NO: 47 - protein, 249 aa, Sorghum bicolor
MNSCRQMELHYINTGFPYTITESFMDFFEGLTYAHADFALMDGFQDQGNPYWAMMHTNSYKYGYSGPGNYYTYAHVYDIDDYMHRADGGRRVWDNTTPANNVDSANVVLQGSEAPRTTANTTTEECIQQVHQSPGSPHVVWQDNIDPDNMTYEELLDLGEVVGTQSRGLSQERISSLPVTKYKCGFFSRKKTRRERCVICQMEYRRGNLQMTLPCKHVYHASCVTRWLSINKVCPVCFAEVPGDEPKRQ

SEQ ID NO: 48 - protein, 253 aa, Zea mays
MNSSRQMELHYINTGFPYTITESFMDFFEGLTYAHADFALTDGFQDQGNPYWAMMHTNSYKYGYSGPGNYYSYAHVYDIDDYMRRADGGRRIWDNTTPVNNVDSANVVLQGGEAPHTTTNTINKECIQQVHQSPGSPQVVWQDNIEPDNMTYEELLDLGEAVGTQSRGLSQERISSLPVTKYKCGFFSRKKTRRERCVICQMEYRRGNLQMTLPCKHVYHASCVTRWLGINKVCPVCFAEVPGEDPEAMSQQL

SEQ ID NO: 49 - protein, 249 aa, Zea mays
MTSSRQMELHYINTGFPYTITESFMDFFEGLTYAHADFALMDGFQDQGNPYWTMMHTNSYKYGYSGSGNYYSYAHAYDIDDYMHRTDGGRRTWDNTTPVNNVDSANVVLQGGEAPRTTANTTSEDCIQQVHQSPGSPQVVWQDNIDPDNMTYEELLDLGEAVGTQSRGLSQECISLLPITKYKCGFFSRKKTRRERCVICQMEYRRGNLQITLPCKHVYHASCVTRWLSINKVCPVCFAEVPGEDSLRQ

SEQ ID NO: 50 - protein, 272 aa, Oryza sativa
MTESHERDTEVTRWQVHDPSEGMNGSRQMELHYINTGFPYTITESFMDFFEGLTYAHADFAIADAFHDQANPYWAMMHTNSYKYGYSGAGNYYSYGHVYDMNDYMHRADGGRRIWDNATPVNNTESPNVVLQGGETPHANTSSTTEECIQQQVHQNSSSPQVIWQDNIDPDNMTYEELLDLGEAVGTQSRGLSQERISLLPVTKYKCGFFSRKKTRRERCVICQMEYRRGNLQMTLPCKHVYHASCVTRWLSINKVCPVCFAEVPGDEPKRQ

SEQ ID NO: 51 - protein, 250 aa, Oryza sativa
MNGSRQMELHYINTGFPYTITESFMDFFEGLTYAHADFAIADAFHDQANPYWAMMHTNSYKYGYSGAGNYYSYGHVYDMNDYMHRADGGRRIWDNATPVNNTESPNVVLQGGETPHANTSSTTEECIQQQVHQNSSSPQVIWQDNIDPDNMTYEELLDLGEAVGTQSRGLSQERISLLPVTKYKCGFFSRKKTRRERCVICQMEYRRGNLQMTLPCKHVYHASCVTRWLSINKVCPVCFAEVPGDEPKRQ

SEQ ID NO: 52 - protein, 251 aa, Brachypodium distachyon
MNGSRQMELHYINTGFPYTITESFMDFFEGLTYAHADFALADAFQDQANPYWTMMQTNSYKYGYSGASNYYSYGHVYDMNDYMHRADGGRRIWDNPTPASNTDSPNVVLQGAAEAPHPRASSTTEECIQQPVHQNSSSPQVVWQDNVDPDNMTYEELLDLGEAVGTQSRGLSQERISSLPVTKYKCGFFSRKKTRRERCVICQMEYRRGDLQMALPCKHVYHASCVTRWLSINKVCPVCFAEVPSEEPSRQ

SEQ ID NO: 53 - protein, 246 aa, Solanum lycopersicum
MNWNQQTEIYYTNGAMPYNSIGSFMDFFGGVTYDHVNYIFADPPYAQESLYPSISTNPYKFGYSEAGSFSYYDYDREYVVNDHVSGIEEHDRHLENPSTTTVNVAANVHREEISGSNSLTNSVECPRGQINTRDSEVVWQDNIDPDNMTYEELLELGEAVGTQSRGLSQNQISLLPVTKFKCGFFSRKKSRKERCVICQMEYKRKDQQVTLPCKHVYHAGCGSRWLSINKACPICYTEVVINTSKR

SEQ ID NO: 54 - protein, 10 aa, Artificial sequence
  Synthetic sequence: LIM domain motif
  VARIANT (2)..(3): Xaa is any amino acid
  VARIANT (5)..(6): Xaa is any amino acid
  VARIANT (8)..(9): Xaa is any amino acid
HXXCXXCXXC